European Patent Application EP 4 606 815 A1, published August 27, 2025. Title: carrier peptide fragment and use thereof. Applicant: TOAGOSEI CO., LTD. The sequence listing filed with the application follows.

SEQUENCE LISTING (1 sequence)

SEQ ID NO: 1 - protein, 8 aa, synthetic construct
KFRAQRRW